European Patent Application EP 4 122 478 A1, published January 25, 2023. Title: COMPOSITIONS AND METHODS FOR USING STAT1/3 INHIBITORS WITH ONCOLYTIC HERPES VIRUS. Applicant: Jia, William Delwar, Zahid. Application WO. The sequence listing filed with the application follows.

SEQUENCE LISTING (16 sequences)

SEQ ID NO: 1 - DNA, 18 bp, Artificial Sequence
  PCR Primer
ggcctgcttccggatctc

SEQ ID NO: 2 - DNA, 21 bp, Artificial Sequence
  PCR Primer
ggtgatgaaggagctgctgtt

SEQ ID NO: 3 - DNA, 21 bp, Artificial Sequence
  PCR Primer
gtctggcggacattaaggaca

SEQ ID NO: 4 - DNA, 20 bp, Artificial Sequence
  PCR Primer
tggccagaatgacaaacacg

SEQ ID NO: 5 - DNA, 19 bp, Artificial Sequence
  PCR Primer
acgaggcccagagcaagag

SEQ ID NO: 6 - DNA, 20 bp, Artificial Sequence
  PCR Primer
tctccatgtcgtcccagttg

SEQ ID NO: 7 - DNA, 18 bp, Artificial Sequence
  PCR Primer
gcgccccatggtcgtgtt

SEQ ID NO: 8 - DNA, 17 bp, Artificial Sequence
  PCR Primer
ctccgccgccgaggttc

SEQ ID NO: 9 - DNA, 17 bp, Artificial Sequence
  PCR Primer
gccgccgcctactaccc

SEQ ID NO: 10 - DNA, 18 bp, Artificial Sequence
  PCR Primer
gctgccgcgactgtgatg

SEQ ID NO: 11 - DNA, 21 bp, Artificial Sequence
  PCR Primer
tgaaccccagccccagaaacc

SEQ ID NO: 12 - DNA, 23 bp, Artificial Sequence
  PCR Primer
tcgagtaaaccatgttaaggacc

SEQ ID NO: 13 - DNA, 21 bp, Artificial Sequence
  PCR Primer
gtctggcggacattaaggaca

SEQ ID NO: 14 - DNA, 20 bp, Artificial Sequence
  PCR Primer
tggccagaatgacaaacacg

SEQ ID NO: 15 - DNA, 19 bp, Artificial Sequence
  PCR Primer
acgaggcccagagcaagag

SEQ ID NO: 16 - DNA, 20 bp, Artificial Sequence
  PCR Primer
tctccatgtcgtcccagttg